European Patent Specification EP 3 870 696 B1, published March 26, 2025. Title: METHODS AND KITS FOR DEPLETION AND ENRICHMENT OF NUCLEIC ACID SEQUENCES. Applicant: University of Washington Rosenberg, Alexander B. Roco, Charles Seelig, Georg. The sequence listing filed with the application follows.

SEQUENCE LISTING (22 sequences)

SEQ ID NO: 1 - DNA, 51 bp, Artificial sequence
  Synthetic
  misc_feature (1)..(51): DNA/RNA Hybrid
  misc_feature (17)..(17): G at position 17 is RNA
  misc_feature (20)..(20): G at position 20 is RNA
  misc_feature (24)..(24): G at position 24 is RNA
aagcagtggtatcaacgcagagtgaatgggtaccaaacgacgagcgtgaca

SEQ ID NO: 2 - DNA, 58 bp, Artificial sequence
  Synthetic
  misc_feature (1)..(58): DNA/RNA Hybrid
  misc_feature (18)..(18): G at position 18 is RNA
  misc_feature (22)..(22): G at position 22 is RNA
  misc_feature (30)..(30): G at position 30 is RNA
gtgactggagttcagacgtgtgctcttccgatctccaatgcttaatcagtgaggcacc

SEQ ID NO: 3 - DNA, 47 bp, Artificial sequence
  Synthetic
  misc_feature (1)..(47): DNA/RNA Hybrid
  misc_feature (17)..(17): G at position 17 is RNA
  misc_feature (20)..(20): G at position 20 is RNA
  misc_feature (24)..(24): G at position 24 is RNA
aagcagtggtatcaacgcagagtgaatgggcccgctgttctgcagcc

SEQ ID NO: 4 - DNA, 53 bp, Artificial sequence
  Synthetic
  misc_feature (1)..(53): DNA/RNA Hybrid
  misc_feature (18)..(18): G at position 18 is RNA
  misc_feature (22)..(22): G at position 22 is RNA
  misc_feature (30)..(30): G at position 30 is RNA
gtgactggagttcagacgtgtgctcttccgatctattcctttgccctcggacg

SEQ ID NO: 5 - DNA, 20 bp, Artificial sequence
  Synthetic
atggcccagtcctctcccaa

SEQ ID NO: 6 - DNA, 22 bp, Artificial sequence
  Synthetic
aggagtaagacccctggaccac

SEQ ID NO: 7 - DNA, 18 bp, Artificial sequence
  Synthetic
agaaccctgaccctgccg

SEQ ID NO: 8 - DNA, 24 bp, Artificial sequence
  Synthetic
ctgaaaaacgtgttcccacccgag

SEQ ID NO: 9 - DNA, 22 bp, Artificial sequence
  Synthetic
acctgaacaaggtgttcccacc

SEQ ID NO: 10 - DNA, 32 bp, Artificial sequence
  Synthetic
  misc_feature (1)..(32): DNA/RNA Hybrid
  misc_feature (16)..(16): G at position 16 is RNA
  misc_feature (18)..(18): G at position 18 is RNA
  misc_feature (20)..(20): G at position 20 is RNA
  misc_feature (28)..(28): G at position 28 is RNA
ttttttttttcagacgtgtgctcttccgatct

SEQ ID NO: 11 - DNA, 33 bp, Artificial sequence
  Synthetic
  misc_feature (1)..(33): DNA/RNA Hybrid
  misc_feature (19)..(19): G at position 19 is RNA
  misc_feature (27)..(27): G at position 27 is RNA
  misc_feature (30)..(30): G at position 30 is RNA
  misc_feature (32)..(32): G at position 32 is RNA
ttttttttttaagcagtggtatcaacgcagagt

SEQ ID NO: 12 - DNA, 23 bp, Artificial sequence
  Synthetic
aagcagtggtatcaacgcagagt

SEQ ID NO: 13 - DNA, 22 bp, Artificial sequence
  Synthetic
cagacgtgtgctcttccgatct

SEQ ID NO: 14 - protein, 130 aa, Aspergillus oryzae
MMYSKLLTLTTLLLPTALALPSLVERACDYTCGSNCYSSSDVSTAQAAGYQLHEDGETVGSNSYPHKYNNYEGFDFSVSSPYYEWPILSSGDVYSGGSPGADRVVFNENNQLAGVITHTGASGNNFVECT

SEQ ID NO: 15 - protein, 150 aa, Bos taurus
MALKSLVLLSLLVLVLLLVRVQPSLGKETAAAKFERQHMDSSTSAASSSNYCNQMMKSRNLTKDRCKPVNTFVHESLADVQAVCSQKNVACKNGQTNCYQSYSTMSITDCRETGSSKYPNCAYKTTQANKHIIVACEGNPYVPVHFDASV

SEQ ID NO: 16 - protein, 198 aa, Escherichia coli
MIEFVYPHTQLVAGVDEVGRGPLVGAVVTAAVILDPARPIAGLNDSKKLSEKRRLALCEEIKEKALSWSLGRAEPHEIDELNILHATMLAMQRAVAGLHIAPEYVLIDGNRCPKLPMPAMAVVKGDSRVPEISAASILAKVTRDAEMAALDIVFPQYGFAQHKGYPTAFHLEKLAEHGATEHHRRSFGPVKRALGLAS

SEQ ID NO: 17 - protein, 155 aa, Escherichia coli
MLKQVEIFTDGSCLGNPGPGGYGAILRYRGREKTFSAGYTRTTNNRMELMAAIVALEALKEHCEVILSTDSQYVRQGITQWIHNWKKRGWKTADKKPVKNVDLWQRLDAALGQHQIKWEWVKGHAGHPENERCDELARAAAMNPTLEDTGYQVEV

SEQ ID NO: 18 - protein, 226 aa, Escherichia coli
MNPIVINRLQRKLGYTFNHQELLQQALTHRSASSKHNERLEFLGDSILSYVIANALYHRFPRVDEGDMSRMRATLVRGNTLAELAREFELGECLRLGPGELKSGGFRRESILADTVEALIGGVFLDSDIQTVEKLILNWYQTRLDEISPGDKQKDPKTRLQEYLQGRHLPLPTYLVVQVRGEAHDQEFTIHCQVSGLSEPVVGTGSSRRKAEQAAAEQALKKLELE

SEQ ID NO: 19 - DNA, 26 bp, Artificial sequence
  Synthetic
acggggagtcaggcaactatggatga

SEQ ID NO: 20 - DNA, 61 bp, Artificial sequence
  Synthetic
  misc_feature (1)..(61): DNA/RNA Hybrid
  misc_feature (27)..(27): G at position 27 is RNA
  misc_feature (30)..(30): G at position 30 is RNA
  misc_feature (34)..(34): G at position 34 is RNA
ttttttttttaagcagtggtatcaacgcagagtgaatgggtaccaaacgacgagcgtgaca

SEQ ID NO: 21 - DNA, 56 bp, Artificial sequence
  Synthetic
  misc_feature (1)..(56): DNA/RNA Hybrid
  misc_feature (16)..(16): G at position 16 is RNA
  misc_feature (20)..(20): G at position 20 is RNA
  misc_feature (28)..(28): G at position 28 is RNA
ttttttttttcagacgtgtgctcttccgatctccaatgcttaatcagtgaggcacc

SEQ ID NO: 22 - DNA, 28 bp, Artificial sequence
  Synthetic
agaagtactcgccgatagtggaaaccga